European Patent Specification EP 3 470 418 B1, published July 31, 2024. Title: Site-specific RI labelled antibody with an IgG binding peptide. Applicant: Kagoshima University. The sequence listing filed with the application follows.

SEQUENCE LISTING (37 sequences)

SEQ ID NO: 1 - protein, 13 aa, Artificial
  IgG-binding peptide
  misc_feature (6)..(6): Xaa is lysine, cystein, aspartic acid, glutamic acid, 2-amino suberic acid, or diaminopropionic acid
DCAYHXGELVWCT

SEQ ID NO: 2 - protein, 17 aa, Artificial
  IgG-binding peptide
  misc_feature (8)..(8): Xaa is lysine, cystein, aspartic acid, glutamic acid, 2-amino suberic acid, or diaminopropionic acid
GPDCAYHXGELVWCTFH

SEQ ID NO: 3 - protein, 13 aa, Artificial
  IgG-binding peptide
  misc_feature (6)..(6): Xaa is lysine, cystein, aspartic acid, glutamic acid, 2-amino suberic acid, or diaminopropionic acid
RCAYHXGELVWCS

SEQ ID NO: 4 - protein, 17 aa, Artificial
  IgG-binding peptide
  misc_feature (8)..(8): Xaa is lysine, cystein, aspartic acid, glutamic acid, 2-amino suberic acid, or diaminopropionic acid
GPRCAYHXGELVWCSFH

SEQ ID NO: 5 - protein, 17 aa, Artificial
  IgG-binding peptide
  misc_feature (8)..(8): Xaa is lysine, cystein, aspartic acid, glutamic acid, 2-amino suberic acid, or diaminopropionic acid
SPDCAYHXGELVWCTFH

SEQ ID NO: 6 - protein, 17 aa, Artificial
  IgG-binding peptide
  misc_feature (8)..(8): Xaa is lysine, cystein, aspartic acid, glutamic acid, 2-amino suberic acid, or diaminopropionic acid
GDDCAYHXGELVWCTFH

SEQ ID NO: 7 - protein, 17 aa, Artificial
  IgG-binding peptide
  misc_feature (8)..(8): Xaa is lysine, cystein, aspartic acid, glutamic acid, 2-amino suberic acid, or diaminopropionic acid
GPSCAYHXGELVWCTFH

SEQ ID NO: 8 - protein, 17 aa, Artificial
  IgG-binding peptide
  misc_feature (8)..(8): Xaa is lysine, cystein, aspartic acid, glutamic acid, 2-amino suberic acid, or diaminopropionic acid
GPDCAYHXGELVWCSFH

SEQ ID NO: 9 - protein, 17 aa, Artificial
  IgG-binding peptide
  misc_feature (8)..(8): Xaa is lysine, cystein, aspartic acid, glutamic acid, 2-amino suberic acid, or diaminopropionic acid
GPDCAYHXGELVWCTHH

SEQ ID NO: 10 - protein, 17 aa, Artificial
  IgG-binding peptide
  misc_feature (8)..(8): Xaa is lysine, cystein, aspartic acid, glutamic acid, 2-amino suberic acid, or diaminopropionic acid
GPDCAYHXGELVWCTFY

SEQ ID NO: 11 - protein, 17 aa, Artificial
  IgG-binding peptide
  misc_feature (8)..(8): Xaa is lysine, cystein, aspartic acid, glutamic acid, 2-amino suberic acid, or diaminopropionic acid
SPDCAYHXGELVWCTFY

SEQ ID NO: 12 - protein, 17 aa, Artificial
  IgG-binding peptide
  misc_feature (8)..(8): Xaa is lysine, cystein, aspartic acid, glutamic acid, 2-amino suberic acid, or diaminopropionic acid
SDDCAYHXGELVWCTFY

SEQ ID NO: 13 - protein, 17 aa, Artificial
  IgG-binding peptide
  misc_feature (8)..(8): Xaa is lysine, cystein, aspartic acid, glutamic acid, 2-amino suberic acid, or diaminopropionic acid
RGNCAYHXGQLVWCTYH

SEQ ID NO: 14 - protein, 13 aa, Artificial
  IgG-binding peptide
  misc_feature (6)..(6): Xaa is lysine, cystein, aspartic acid, glutamic acid, 2-amino suberic acid, or diaminopropionic acid
DCTYHXGNLVWCT

SEQ ID NO: 15 - protein, 13 aa, Artificial
  IgG-binding peptide
  misc_feature (6)..(6): Xaa is lysine, cystein, aspartic acid, glutamic acid, 2-amino suberic acid, or diaminopropionic acid
DCAYHXGNLVWCT

SEQ ID NO: 16 - protein, 13 aa, Artificial
  IgG-binding peptide
  misc_feature (6)..(6): Xaa is lysine, cystein, aspartic acid, glutamic acid, 2-amino suberic acid, or diaminopropionic acid
DCTYHXGELVWCT

SEQ ID NO: 17 - protein, 13 aa, Artificial
  IgG-binding peptide
  misc_feature (6)..(6): Xaa is lysine, cystein, aspartic acid, glutamic acid, 2-amino suberic acid, or diaminopropionic acid
DCAWHXGELVWCT

SEQ ID NO: 18 - protein, 13 aa, Artificial
  IgG-binding peptide
  misc_feature (6)..(6): Xaa is lysine, cystein, aspartic acid, glutamic acid, 2-amino suberic acid, or diaminopropionic acid
DCTYTXGNLVWCT

SEQ ID NO: 19 - protein, 13 aa, Artificial
  IgG-binding peptide
  misc_feature (6)..(6): Xaa is lysine, cystein, aspartic acid, glutamic acid, 2-amino suberic acid, or diaminopropionic acid
DCAYTXGNLVWCT

SEQ ID NO: 20 - protein, 13 aa, Artificial
  IgG-binding peptide
  misc_feature (6)..(6): Xaa is lysine, cystein, aspartic acid, glutamic acid, 2-amino suberic acid, or diaminopropionic acid
DCSYTXGNLVWCT

SEQ ID NO: 21 - protein, 13 aa, Artificial
  IgG-binding peptide
  misc_feature (6)..(6): Xaa is lysine, cystein, aspartic acid, glutamic acid, 2-amino suberic acid, or diaminopropionic acid
DCTWTXGNLVWCT

SEQ ID NO: 22 - protein, 13 aa, Artificial
  IgG-binding peptide
  misc_feature (6)..(6): Xaa is lysine, cystein, aspartic acid, glutamic acid, 2-amino suberic acid, or diaminopropionic acid
DCTYHXGNLVWCT

SEQ ID NO: 23 - protein, 13 aa, Artificial
  IgG-binding peptide
  misc_feature (6)..(6): Xaa is lysine, cystein, aspartic acid, glutamic acid, 2-amino suberic acid, or diaminopropionic acid
DCTYRXGNLVWCT

SEQ ID NO: 24 - protein, 13 aa, Artificial
  IgG-binding peptide
  misc_feature (6)..(6): Xaa is lysine, cystein, aspartic acid, glutamic acid, 2-amino suberic acid, or diaminopropionic acid
DCTYSXGNLVWCT

SEQ ID NO: 25 - protein, 13 aa, Artificial
  IgG-binding peptide
  misc_feature (6)..(6): Xaa is lysine, cystein, aspartic acid, glutamic acid, 2-amino suberic acid, or diaminopropionic acid
DCTYTXGNLVWCT

SEQ ID NO: 26 - protein, 13 aa, Artificial
  IgG-binding peptide
  misc_feature (6)..(6): Xaa is lysine, cystein, aspartic acid, glutamic acid, 2-amino suberic acid, or diaminopropionic acid
DCTYTXGELVWCT

SEQ ID NO: 27 - protein, 13 aa, Artificial
  IgG-binding peptide
  misc_feature (6)..(6): Xaa is lysine, cystein, aspartic acid, glutamic acid, 2-amino suberic acid, or diaminopropionic acid
DCTYTXGRLVWCT

SEQ ID NO: 28 - protein, 13 aa, Artificial
  IgG-binding peptide
  misc_feature (6)..(6): Xaa is lysine, cystein, aspartic acid, glutamic acid, 2-amino suberic acid, or diaminopropionic acid
DCTYTXGDLVWCT

SEQ ID NO: 29 - protein, 13 aa, Artificial
  IgG-binding peptide
  misc_feature (6)..(6): Xaa is lysine, cystein, aspartic acid, glutamic acid, 2-amino suberic acid, or diaminopropionic acid
DCTYTXGNLIWCT

SEQ ID NO: 30 - protein, 110 aa, Homo Sapiens
APELLGGPSVFLFPPKPKDTLMISRTPEVTCVVVDVSHEDPEVKFNWYVDGVEVHNAKTKPREEQYNSTYRVVSVLTVLHQDWLNGKEYKCKVSNKALPAPIEKTISKAK

SEQ ID NO: 31 - protein, 17 aa, Artificial
  IgG-binding peptide
  misc_feature (2)..(2): Xaa is homocysteine
  misc_feature (16)..(16): Xaa is homocysteine
GXDCAYHRGELVWCTXH

SEQ ID NO: 32 - protein, 17 aa, Artificial
  IgG-binding peptide
  misc_feature (8)..(8): Xaa is lysine, cystein, aspartic acid, glutamic acid, 2-amino suberic acid, or diaminopropionic acid
GPDCAYHXGELVWCTFH

SEQ ID NO: 33 - protein, 13 aa, Artificial
  IgG-binding peptide
DCAYHRGELVWCT

SEQ ID NO: 34 - protein, 13 aa, Artificial
  IgG-binding peptide
DCAYHKGELVWCT

SEQ ID NO: 35 - protein, 17 aa, Artificial
  IgG-binding peptide
  misc_feature (8)..(8): Xaa is lysine, cystein, aspartic acid, glutamic acid, 2-amino suberic acid, or diaminopropionic acid
RGNCAYHXGQLVWCTYH

SEQ ID NO: 36 - protein, 17 aa, Artificial
  IgG-binding peptide
  misc_feature (2)..(2): Xaa is homocysteine
  misc_feature (8)..(8): Xaa is lysine, cystein, aspartic acid, glutamic acid, 2-amino suberic acid, or diaminopropionic acid
  misc_feature (16)..(16): Xaa is homocysteine
GXDCAYHXGELVWCTXH

SEQ ID NO: 37 - protein, 17 aa, Artificial
  IgG-binding peptide
GPDCAYHKGELVWCTFH